European Patent Application EP 4 342 907 A1, published March 27, 2024. Title: Switchable chimeric antigen receptors and their use. Applicant: AvenCell Therapeutics Inc. The sequence listing filed with the application follows.

SEQUENCE LISTING (61 sequences)

SEQ ID NO: 1 - protein, 33 aa, Saccharomyces cerevisiae
RMKQLEPKVEELLPKNYHLENEVARLKKLVGER

SEQ ID NO: 2 - protein, 14 aa, Saccharomyces cerevisiae
NYHLENEVARLKKL

SEQ ID NO: 3 - protein, 51 aa, Homo sapiens
MDPDLEIRAAFLRQRNTALRTEVAELEQEVQRLENEVSQYETRYGPLGGGK

SEQ ID NO: 4 - protein, 51 aa, Homo sapiens
MDPDLEIEAAFLERENTALETRVAELRQRVQRLRNRVSQYRTRYGPLGGGK

SEQ ID NO: 5 - protein, 10 aa, Homo sapiens
KPLPEVTDEY

SEQ ID NO: 6 - protein, 20 aa, Homo sapiens
  VARIANT 16: note = X can be any amino acid
LEKEALKKIIEDQQEXLNKW

SEQ ID NO: 7 - protein, 20 aa, Homo sapiens
LEKEALKKIIEDQQEALNKW

SEQ ID NO: 8 - protein, 113 aa, synthetic construct
  source 1..113: note = Humanized scFv VL chain
  VARIANT 24: note = X can be any amino acid
  VARIANT 35: note = X can be any amino acid
  VARIANT 61: note = X can be any amino acid
  VARIANT 101: note = X can be any amino acid
DIVMTQSPDSLAVSLGERATINCXSSQSLLNSRTXKNYLAWYQQKPGQPPKLLIYWASTRXSGVPDRFSGSGSGTDFTLTISSLQAEDVAVYYCKQSYNLXTFGGGTKVEILK

SEQ ID NO: 9 - protein, 120 aa, synthetic construct
  source 1..120: note = Humanized scFv VH chain
QVQLVQSGAEVKKPGASVKVSCKASGYTFTHYYIYWVRQAPGQGLEWMGGVNPSNGGTHFNEKFKSRVTMTRDTSISTAYMELSRLRSDDTAVYYCARSEYDYGLGFAYWGQGTLVTVSS

SEQ ID NO: 10 - protein, 112 aa, synthetic construct
  source 1..112: note = Humanized scFv VL chain
DIVMTQSPDSLAVSLGERATINCKSSQSLLNSRTPKNYLAWYQQKPGQPPKLLIYWASTRKSGVPDRFSGSGSGTDFTLTISSLQAEDVAVYYCKQSYNLLTFGGGTKVEIK

SEQ ID NO: 11 - protein, 118 aa, synthetic construct
  source 1..118: note = Humanized scFv VH chain
EVQLVESGGGLVQPGGSLRLSCAASGFTFSDFWMNWVRQAPGKGLEWVGQIRNKPNNYETYYSDSLKGRFTISRDDSKSITYLQMNSLRAEDTAVYYCTLGNSWFAYWGQGTLVTVSS

SEQ ID NO: 12 - protein, 112 aa, synthetic construct
  source 1..112: note = Humanized scFv VL chain
DIVMTQSPDSLAVSLGERATINCRSSQSLLDSRTKKNYLAWYQQKPGQPPKLLIYWASTRESGVPDRFSGSGSGTDFTLTISSLQAEDVAVYYCKQSYNLPTFGGGTKVEIK

SEQ ID NO: 13 - protein, 5 aa, synthetic construct
  source 1..5: note = linker
GGGGS

SEQ ID NO: 14 - protein, 25 aa, synthetic construct
  source 1..25: note = linker
GGGGSGGGGSGGGGSGGGGSGGGGS

SEQ ID NO: 15 - protein, 25 aa, synthetic construct
  source 1..25: note = linker
GGGGSGGGGSGASAAGGGGSGGGGS

SEQ ID NO: 16 - protein, 133 aa, synthetic construct
  source 1..133: note = CD28 extracellular hinge domain with mutation
KILVKQSPMLVAYDNAVNLSCKYSYNLFSREFRASLHKGLDSAVEVCVVYGNYSQQLQVYSKTGFNCDGKLGNESVTFYLQNLYVNQTDIYFCKIEVMAPPPALDNEKSNGTIIHVKGKHLCPSPLFPGPSKP

SEQ ID NO: 17 - protein, 27 aa, Homo sapiens
FWVLVVVGGVLACYSLLVTVAFIIFWV

SEQ ID NO: 18 - protein, 21 aa, Homo sapiens
FWLPIGCAAFVVVCILGCILI

SEQ ID NO: 19 - protein, 41 aa, synthetic construct
  source 1..41: note = CD28 intracellular signaling domain with mutations
RSKRSRGGHSDYMNMTPRRPGPTRKHYQPYAPPRDFAAYRS

SEQ ID NO: 20 - protein, 41 aa, synthetic construct
  source 1..41: note = CD28 intracellular signaling domain with mutations
RSKRSRGGHSDYMFMTPRRPGPTRKHYQPYAPPRDFAAYRS

SEQ ID NO: 21 - protein, 109 aa, Homo sapiens
FSRSADAPAYQQGQNQLYNELNLGRREEYDVLDKRRGRDPEMGGKPRRKNPQEGLYNELQKDKMAEAYSEIGMKGERRRGKGHDGLYQGLSTATKDTYDALHMQALPPR

SEQ ID NO: 22 - protein, 109 aa, synthetic construct
  source 1..109: note = CD3zeta intracellular signaling domain with mutation
FSRSADAPAYQQGQNQLYNELNLGRREEYDVLDKRRGRDPEMGGKPRRKNPQEGLYNELQKDKMAEAYSEIGMKGERRRGKGHDGLYQGLSTATKDTYGALHMQALPPR

SEQ ID NO: 23 - protein, 112 aa, synthetic construct
  source 1..112: note = CD3zeta intracellular signaling domain with mutations
RVKFSRSADAPAYQQGQNQLYNELNLGRREEYDVLDKRRGRDPEMGGKPRRKNPQEGLYNELQKDKMAEAYSEIGMKGERRRGKGHDGLYQGLSTATKDTYDAYRHQALPPR

SEQ ID NO: 24 - protein, 38 aa, Homo sapiens
CWLTKKKYSSSVHDPNGEYMFMRAVNTAKKSRLTDVTL

SEQ ID NO: 25 - protein, 42 aa, Homo sapiens
KRGRKKLLYIFKQPFMRPVQTTQEEDGCSCRFPEEEEGGCEL

SEQ ID NO: 26 - protein, 155 aa, synthetic construct
  source 1..155: note = truncated IL-7Ralpha intracellular signaling domain
KKRIKPIVWPSLPDHKKTLEHLCKKPRKNLNVSFNPESFLDCQIHRVDDIQARDEVEGFLQDTFPQQLEESEKQRLGGDVQSPNCPSEDVVIGPHVYQDLLLSLGTTNSTLPPPFSLQSGILTLNPVAQGQPILTSLGSNQEEAYVTMSSFYQNQ

SEQ ID NO: 27 - protein, 94 aa, synthetic construct
  source 1..94: note = truncated IL-2Rbeta intracellular signaling domain
NCRNTGPWLKKVLKCNTPDPSKFFSQLSSEHGGDVQKWLSSPFPSSSFSPGGLAPEISPLEVLERDKVTQLLPLNTDAYLSLQELQGQDPTHLV

SEQ ID NO: 28 - protein, 634 aa, synthetic construct
  source 1..634: note = humanized homo sapiens/mus musculus chimera
MRRMQLLLLIALSLALVTNSEFKPLPEVTDEYAAAGPGGGGSKILVKQSPMLVAYDNAVNLSCKYSYNLFSREFRASLHKGLDSAVEVCVVYGNYSQQLQVYSKTGFNCDGKLGNESVTFYLQNLYVNQTDIYFCKIEVMAPPPALDNEKSNGTIIHVKGKHLCPSPLFPGPSKPFWVLVVVGGVLACYSLLVTVAFIIFWVRSKRSRGGHSDYMNMTPRRPGPTRKHYQPYAPPRDFAAYRSGGGGSGGGASGGGGSFSRSADAPAYQQGQNQLYNELNLGRREEYDVLDKRRGRDPEMGGKPRRKNPQEGLYNELQKDKMAEAYSEIGMKGERRRGKGHDGLYQGLSTATKDTYGALHMQALPPRGSGSSGEGRGSLLTCGDVEENPGPPVATMVSKGEELFTGVVPILVELDGDVNGHKFSVSGEGEGDATYGKLTLKFICTTGKLPVPWPTLVTTLTYGVQCFSRYPDHMKQHDFFKSAMPEGYVQERTIFFKDDGNYKTRAEVKFEGDTLVNRIELKGIDFKEDGNILGHKLEYNYNSHNVYIMADKQKNGIKVNFKIRHNIEDGSVQLADHYQQNTPIGDGPVLLPDNHYLSTQSALSKDPNEKRDHMVLLEFVTAAGITLGMDELYK

SEQ ID NO: 29 - protein, 624 aa, synthetic construct
  source 1..624: note = humanized homo sapiens/mus musculus chimera
MRRMQLLLLIALSLALVTNSEFKPLPEVTDEYAAAGPGGGGSKILVKQSPMLVAYDNAVNLSCKYSYNLFSREFRASLHKGLDSAVEVCVVYGNYSQQLQVYSKTGFNCDGKLGNESVTFYLQNLYVNQTDIYFCKIEVMAPPPALDNEKSNGTIIHVKGKHLCPSPLFPGPSKPFWVLVVVGGVLACYSLLVTVAFIIFWVRSKRSRGGHSDYMNMTPRRPGPTRKHYQPYAPPRDFAAYRSGGGGSFSRSADAPAYQQGQNQLYNELNLGRREEYDVLDKRRGRDPEMGGKPRRKNPQEGLYNELQKDKMAEAYSEIGMKGERRRGKGHDGLYQGLSTATKDTYDALHMQALPPRGSGSSGEGRGSLLTCGDVEENPGPPVATMVSKGEELFTGVVPILVELDGDVNGHKFSVSGEGEGDATYGKLTLKFICTTGKLPVPWPTLVTTLTYGVQCFSRYPDHMKQHDFFKSAMPEGYVQERTIFFKDDGNYKTRAEVKFEGDTLVNRIELKGIDFKEDGNILGHKLEYNYNSHNVYIMADKQKNGIKVNFKIRHNIEDGSVQLADHYQQNTPIGDGPVLLPDNHYLSTQSALSKDPNEKRDHMVLLEFVTAAGITLGMDELYK

SEQ ID NO: 30 - protein, 671 aa, synthetic construct
  source 1..671: note = humanized homo sapiens/mus musculus chimera
MRRMQLLLLIALSLALVTNSEFKPLPEVTDEYAAAGPGGGGSKILVKQSPMLVAYDNAVNLSCKYSYNLFSREFRASLHKGLDSAVEVCVVYGNYSQQLQVYSKTGFNCDGKLGNESVTFYLQNLYVNQTDIYFCKIEVMAPPPALDNEKSNGTIIHVKGKHLCPSPLFPGPSKPFWVLVVVGGVLACYSLLVTVAFIIFWVRSKRSRGGHSDYMNMTPRRPGPTRKHYQPYAPPRDFAAYRSGGGGSKRGRKKLLYIFKQPFMRPVQTTQEEDGCSCRFPEEEEGGCELGGGGSFSRSADAPAYQQGQNQLYNELNLGRREEYDVLDKRRGRDPEMGGKPRRKNPQEGLYNELQKDKMAEAYSEIGMKGERRRGKGHDGLYQGLSTATKDTYDALHMQALPPRGSGSSGEGRGSLLTCGDVEENPGPPVATMVSKGEELFTGVVPILVELDGDVNGHKFSVSGEGEGDATYGKLTLKFICTTGKLPVPWPTLVTTLTYGVQCFSRYPDHMKQHDFFKSAMPEGYVQERTIFFKDDGNYKTRAEVKFEGDTLVNRIELKGIDFKEDGNILGHKLEYNYNSHNVYIMADKQKNGIKVNFKIRHNIEDGSVQLADHYQQNTPIGDGPVLLPDNHYLSTQSALSKDPNEKRDHMVLLEFVTAAGITLGMDELYK

SEQ ID NO: 31 - protein, 716 aa, synthetic construct
  source 1..716: note = humanized homo sapiens/mus musculus chimera
MRRMQLLLLIALSLALVTNSEFKPLPEVTDEYAAAGPGGGGSKILVKQSPMLVAYDNAVNLSCKYSYNLFSREFRASLHKGLDSAVEVCVVYGNYSQQLQVYSKTGFNCDGKLGNESVTFYLQNLYVNQTDIYFCKIEVMAPPPALDNEKSNGTIIHVKGKHLCPSPLFPGPSKPFWVLVVVGGVLACYSLLVTVAFIIFWVRSKRSRGGHSDYMNMTPRRPGPTRKHYQPYAPPRDFAAYRSNCRNTGPWLKKVLKCNTPDPSKFFSQLSSEHGGDVQKWLSSPFPSSSFSPGGLAPEISPLEVLERDKVTQLLPLNTDAYLSLQELQGQDPTHLVRVKFSRSADAPAYQQGQNQLYNELNLGRREEYDVLDKRRGRDPEMGGKPRRKNPQEGLYNELQKDKMAEAYSEIGMKGERRRGKGHDGLYQGLSTATKDTYDAYRHQALPPRGSGSSGEGRGSLLTCGDVEENPGPPVATMVSKGEELFTGVVPILVELDGDVNGHKFSVSGEGEGDATYGKLTLKFICTTGKLPVPWPTLVTTLTYGVQCFSRYPDHMKQHDFFKSAMPEGYVQERTIFFKDDGNYKTRAEVKFEGDTLVNRIELKGIDFKEDGNILGHKLEYNYNSHNVYIMADKQKNGIKVNFKIRHNIEDGSVQLADHYQQNTPIGDGPVLLPDNHYLSTQSALSKDPNEKRDHMVLLEFVTAAGITLGMDELYK

SEQ ID NO: 32 - protein, 784 aa, synthetic construct
  source 1..784: note = humanized homo sapiens/mus musculus chimera
MRRMQLLLLIALSLALVTNSEFKPLPEVTDEYAAAGPGGGGSKILVKQSPMLVAYDNAVNLSCKYSYNLFSREFRASLHKGLDSAVEVCVVYGNYSQQLQVYSKTGFNCDGKLGNESVTFYLQNLYVNQTDIYFCKIEVMAPPPALDNEKSNGTIIHVKGKHLCPSPLFPGPSKPFWVLVVVGGVLACYSLLVTVAFIIFWVRSKRSRGGHSDYMNMTPRRPGPTRKHYQPYAPPRDFAAYRSGGGGSKKRIKPIVWPSLPDHKKTLEHLCKKPRKNLNVSFNPESFLDCQIHRVDDIQARDEVEGFLQDTFPQQLEESEKQRLGGDVQSPNCPSEDVVIGPHVYQDLLLSLGTTNSTLPPPFSLQSGILTLNPVAQGQPILTSLGSNQEEAYVTMSSFYQNQGGGGSFSRSADAPAYQQGQNQLYNELNLGRREEYDVLDKRRGRDPEMGGKPRRKNPQEGLYNELQKDKMAEAYSEIGMKGERRRGKGHDGLYQGLSTATKDTYDALHMQALPPRGSGSSGEGRGSLLTCGDVEENPGPPVATMVSKGEELFTGVVPILVELDGDVNGHKFSVSGEGEGDATYGKLTLKFICTTGKLPVPWPTLVTTLTYGVQCFSRYPDHMKQHDFFKSAMPEGYVQERTIFFKDDGNYKTRAEVKFEGDTLVNRIELKGIDFKEDGNILGHKLEYNYNSHNVYIMADKQKNGIKVNFKIRHNIEDGSVQLADHYQQNTPIGDGPVLLPDNHYLSTQSALSKDPNEKRDHMVLLEFVTAAGITLGMDELYK

SEQ ID NO: 33 - protein, 784 aa, synthetic construct
  source 1..784: note = humanized homo sapiens/mus musculus chimera
MRRMQLLLLIALSLALVTNSEFKPLPEVTDEYAAAGPGGGGSKILVKQSPMLVAYDNAVNLSCKYSYNLFSREFRASLHKGLDSAVEVCVVYGNYSQQLQVYSKTGFNCDGKLGNESVTFYLQNLYVNQTDIYFCKIEVMAPPPALDNEKSNGTIIHVKGKHLCPSPLFPGPSKPFWVLVVVGGVLACYSLLVTVAFIIFWVRSKRSRGGHSDYMNMTPRRPGPTRKHYQPYAPPRDFAAYRSGGGGSFSRSADAPAYQQGQNQLYNELNLGRREEYDVLDKRRGRDPEMGGKPRRKNPQEGLYNELQKDKMAEAYSEIGMKGERRRGKGHDGLYQGLSTATKDTYDALHMQALPPRGGGGSKKRIKPIVWPSLPDHKKTLEHLCKKPRKNLNVSFNPESFLDCQIHRVDDIQARDEVEGFLQDTFPQQLEESEKQRLGGDVQSPNCPSEDVVIGPHVYQDLLLSLGTTNSTLPPPFSLQSGILTLNPVAQGQPILTSLGSNQEEAYVTMSSFYQNQGSGSSGEGRGSLLTCGDVEENPGPPVATMVSKGEELFTGVVPILVELDGDVNGHKFSVSGEGEGDATYGKLTLKFICTTGKLPVPWPTLVTTLTYGVQCFSRYPDHMKQHDFFKSAMPEGYVQERTIFFKDDGNYKTRAEVKFEGDTLVNRIELKGIDFKEDGNILGHKLEYNYNSHNVYIMADKQKNGIKVNFKIRHNIEDGSVQLADHYQQNTPIGDGPVLLPDNHYLSTQSALSKDPNEKRDHMVLLEFVTAAGITLGMDELYK

SEQ ID NO: 34 - protein, 624 aa, synthetic construct
  source 1..624: note = humanized homo sapiens/mus musculus chimera
MRRMQLLLLIALSLALVTNSEFKPLPEVTDEYAAAGPGGGGSKILVKQSPMLVAYDNAVNLSCKYSYNLFSREFRASLHKGLDSAVEVCVVYGNYSQQLQVYSKTGFNCDGKLGNESVTFYLQNLYVNQTDIYFCKIEVMAPPPALDNEKSNGTIIHVKGKHLCPSPLFPGPSKPFWVLVVVGGVLACYSLLVTVAFIIFWVRSKRSRGGHSDYMFMTPRRPGPTRKHYQPYAPPRDFAAYRSGGGGSFSRSADAPAYQQGQNQLYNELNLGRREEYDVLDKRRGRDPEMGGKPRRKNPQEGLYNELQKDKMAEAYSEIGMKGERRRGKGHDGLYQGLSTATKDTYDALHMQALPPRGSGSSGEGRGSLLTCGDVEENPGPPVATMVSKGEELFTGVVPILVELDGDVNGHKFSVSGEGEGDATYGKLTLKFICTTGKLPVPWPTLVTTLTYGVQCFSRYPDHMKQHDFFKSAMPEGYVQERTIFFKDDGNYKTRAEVKFEGDTLVNRIELKGIDFKEDGNILGHKLEYNYNSHNVYIMADKQKNGIKVNFKIRHNIEDGSVQLADHYQQNTPIGDGPVLLPDNHYLSTQSALSKDPNEKRDHMVLLEFVTAAGITLGMDELYK

SEQ ID NO: 35 - protein, 662 aa, synthetic construct
  source 1..662: note = humanized homo sapiens/mus musculus chimera
MRRMQLLLLIALSLALVTNSEFKPLPEVTDEYAAAGPGGGGSKILVKQSPMLVAYDNAVNLSCKYSYNLFSREFRASLHKGLDSAVEVCVVYGNYSQQLQVYSKTGFNCDGKLGNESVTFYLQNLYVNQTDIYFCKIEVMAPPPALDNEKSNGTIIHVKGKHLCPSPLFPGPSKPFWLPIGCAAFVVVCILGCILICWLTKKKYSSSVHDPNGEYMFMRAVNTAKKSRLTDVTLGGGGSKRGRKKLLYIFKQPFMRPVQTTQEEDGCSCRFPEEEEGGCELGGGGSFSRSADAPAYQQGQNQLYNELNLGRREEYDVLDKRRGRDPEMGGKPRRKNPQEGLYNELQKDKMAEAYSEIGMKGERRRGKGHDGLYQGLSTATKDTYDALHMQALPPRGSGSSGEGRGSLLTCGDVEENPGPPVATMVSKGEELFTGVVPILVELDGDVNGHKFSVSGEGEGDATYGKLTLKFICTTGKLPVPWPTLVTTLTYGVQCFSRYPDHMKQHDFFKSAMPEGYVQERTIFFKDDGNYKTRAEVKFEGDTLVNRIELKGIDFKEDGNILGHKLEYNYNSHNVYIMADKQKNGIKVNFKIRHNIEDGSVQLADHYQQNTPIGDGPVLLPDNHYLSTQSALSKDPNEKRDHMVLLEFVTAAGITLGMDELYK

SEQ ID NO: 36 - protein, 615 aa, synthetic construct
  source 1..615: note = humanized homo sapiens/mus musculus chimera
MRRMQLLLLIALSLALVTNSEFKPLPEVTDEYAAAGPGGGGSKILVKQSPMLVAYDNAVNLSCKYSYNLFSREFRASLHKGLDSAVEVCVVYGNYSQQLQVYSKTGFNCDGKLGNESVTFYLQNLYVNQTDIYFCKIEVMAPPPALDNEKSNGTIIHVKGKHLCPSPLFPGPSKPFWLPIGCAAFVVVCILGCILICWLTKKKYSSSVHDPNGEYMFMRAVNTAKKSRLTDVTLGGGGSFSRSADAPAYQQGQNQLYNELNLGRREEYDVLDKRRGRDPEMGGKPRRKNPQEGLYNELQKDKMAEAYSEIGMKGERRRGKGHDGLYQGLSTATKDTYDALHMQALPPRGSGSSGEGRGSLLTCGDVEENPGPPVATMVSKGEELFTGVVPILVELDGDVNGHKFSVSGEGEGDATYGKLTLKFICTTGKLPVPWPTLVTTLTYGVQCFSRYPDHMKQHDFFKSAMPEGYVQERTIFFKDDGNYKTRAEVKFEGDTLVNRIELKGIDFKEDGNILGHKLEYNYNSHNVYIMADKQKNGIKVNFKIRHNIEDGSVQLADHYQQNTPIGDGPVLLPDNHYLSTQSALSKDPNEKRDHMVLLEFVTAAGITLGMDELYK

SEQ ID NO: 37 - protein, 894 aa, synthetic construct
  source 1..894: note = humanized homo sapiens/mus musculus chimera
MRRMQLLLLIALSLALVTNSEFQVQLVQSGAEVKKPGASVKVSCKASGYTFTHYYIYWVRQAPGQGLEWMGGVNPSNGGTHFNEKFKSRVTMTRDTSISTAYMELSRLRSDDTAVYYCARSEYDYGLGFAYWGQGTLVTVSSGGGGSGGGGSGGGGSDIVMTQSPDSLAVSLGERATINCKSSQSLLNSRTPKNYLAWYQQKPGQPPKLLIYWASTRKSGVPDRFSGSGSGTDFTLTISSLQAEDVAVYYCKQSYNLLTFGGGTKVEIKAAALEKEALKKIIEDQQEALNKWAAAGPGGGGSKILVKQSPMLVAYDNAVNLSCKYSYNLFSREFRASLHKGLDSAVEVCVVYGNYSQQLQVYSKTGFNCDGKLGNESVTFYLQNLYVNQTDIYFCKIEVMAPPPALDNEKSNGTIIHVKGKHLCPSPLFPGPSKPFWVLVVVGGVLACYSLLVTVAFIIFWVRSKRSRGGHSDYMNMTPRRPGPTRKHYQPYAPPRDFAAYRSGGGGSGGGASGGGGSFSRSADAPAYQQGQNQLYNELNLGRREEYDVLDKRRGRDPEMGGKPRRKNPQEGLYNELQKDKMAEAYSEIGMKGERRRGKGHDGLYQGLSTATKDTYGALHMQALPPRGSGSSGEGRGSLLTCGDVEENPGPPVATMVSKGEELFTGVVPILVELDGDVNGHKFSVSGEGEGDATYGKLTLKFICTTGKLPVPWPTLVTTLTYGVQCFSRYPDHMKQHDFFKSAMPEGYVQERTIFFKDDGNYKTRAEVKFEGDTLVNRIELKGIDFKEDGNILGHKLEYNYNSHNVYIMADKQKNGIKVNFKIRHNIEDGSVQLADHYQQNTPIGDGPVLLPDNHYLSTQSALSKDPNEKRDHMVLLEFVTAAGITLGMDELYK

SEQ ID NO: 38 - protein, 884 aa, synthetic construct
  source 1..884: note = humanized homo sapiens/mus musculus chimera
MRRMQLLLLIALSLALVTNSEFQVQLVQSGAEVKKPGASVKVSCKASGYTFTHYYIYWVRQAPGQGLEWMGGVNPSNGGTHFNEKFKSRVTMTRDTSISTAYMELSRLRSDDTAVYYCARSEYDYGLGFAYWGQGTLVTVSSGGGGSGGGGSGGGGSDIVMTQSPDSLAVSLGERATINCKSSQSLLNSRTPKNYLAWYQQKPGQPPKLLIYWASTRKSGVPDRFSGSGSGTDFTLTISSLQAEDVAVYYCKQSYNLLTFGGGTKVEIKAAALEKEALKKIIEDQQEALNKWAAAGPGGGGSKILVKQSPMLVAYDNAVNLSCKYSYNLFSREFRASLHKGLDSAVEVCVVYGNYSQQLQVYSKTGFNCDGKLGNESVTFYLQNLYVNQTDIYFCKIEVMAPPPALDNEKSNGTIIHVKGKHLCPSPLFPGPSKPFWVLVVVGGVLACYSLLVTVAFIIFWVRSKRSRGGHSDYMNMTPRRPGPTRKHYQPYAPPRDFAAYRSGGGGSFSRSADAPAYQQGQNQLYNELNLGRREEYDVLDKRRGRDPEMGGKPRRKNPQEGLYNELQKDKMAEAYSEIGMKGERRRGKGHDGLYQGLSTATKDTYDALHMQALPPRGSGSSGEGRGSLLTCGDVEENPGPPVATMVSKGEELFTGVVPILVELDGDVNGHKFSVSGEGEGDATYGKLTLKFICTTGKLPVPWPTLVTTLTYGVQCFSRYPDHMKQHDFFKSAMPEGYVQERTIFFKDDGNYKTRAEVKFEGDTLVNRIELKGIDFKEDGNILGHKLEYNYNSHNVYIMADKQKNGIKVNFKIRHNIEDGSVQLADHYQQNTPIGDGPVLLPDNHYLSTQSALSKDPNEKRDHMVLLEFVTAAGITLGMDELYK

SEQ ID NO: 39 - protein, 931 aa, synthetic construct
  source 1..931: note = humanized homo sapiens/mus musculus chimera
MRRMQLLLLIALSLALVTNSEFQVQLVQSGAEVKKPGASVKVSCKASGYTFTHYYIYWVRQAPGQGLEWMGGVNPSNGGTHFNEKFKSRVTMTRDTSISTAYMELSRLRSDDTAVYYCARSEYDYGLGFAYWGQGTLVTVSSGGGGSGGGGSGGGGSDIVMTQSPDSLAVSLGERATINCKSSQSLLNSRTPKNYLAWYQQKPGQPPKLLIYWASTRKSGVPDRFSGSGSGTDFTLTISSLQAEDVAVYYCKQSYNLLTFGGGTKVEIKAAALEKEALKKIIEDQQEALNKWAAAGPGGGGSKILVKQSPMLVAYDNAVNLSCKYSYNLFSREFRASLHKGLDSAVEVCVVYGNYSQQLQVYSKTGFNCDGKLGNESVTFYLQNLYVNQTDIYFCKIEVMAPPPALDNEKSNGTIIHVKGKHLCPSPLFPGPSKPFWVLVVVGGVLACYSLLVTVAFIIFWVRSKRSRGGHSDYMNMTPRRPGPTRKHYQPYAPPRDFAAYRSGGGGSKRGRKKLLYIFKQPFMRPVQTTQEEDGCSCRFPEEEEGGCELGGGGSFSRSADAPAYQQGQNQLYNELNLGRREEYDVLDKRRGRDPEMGGKPRRKNPQEGLYNELQKDKMAEAYSEIGMKGERRRGKGHDGLYQGLSTATKDTYDALHMQALPPRGSGSSGEGRGSLLTCGDVEENPGPPVATMVSKGEELFTGVVPILVELDGDVNGHKFSVSGEGEGDATYGKLTLKFICTTGKLPVPWPTLVTTLTYGVQCFSRYPDHMKQHDFFKSAMPEGYVQERTIFFKDDGNYKTRAEVKFEGDTLVNRIELKGIDFKEDGNILGHKLEYNYNSHNVYIMADKQKNGIKVNFKIRHNIEDGSVQLADHYQQNTPIGDGPVLLPDNHYLSTQSALSKDPNEKRDHMVLLEFVTAAGITLGMDELYK

SEQ ID NO: 40 - protein, 976 aa, synthetic construct
  source 1..976: note = humanized homo sapiens/mus musculus chimera
MRRMQLLLLIALSLALVTNSEFQVQLVQSGAEVKKPGASVKVSCKASGYTFTHYYIYWVRQAPGQGLEWMGGVNPSNGGTHFNEKFKSRVTMTRDTSISTAYMELSRLRSDDTAVYYCARSEYDYGLGFAYWGQGTLVTVSSGGGGSGGGGSGGGGSDIVMTQSPDSLAVSLGERATINCKSSQSLLNSRTPKNYLAWYQQKPGQPPKLLIYWASTRKSGVPDRFSGSGSGTDFTLTISSLQAEDVAVYYCKQSYNLLTFGGGTKVEIKAAALEKEALKKIIEDQQEALNKWAAAGPGGGGSKILVKQSPMLVAYDNAVNLSCKYSYNLFSREFRASLHKGLDSAVEVCVVYGNYSQQLQVYSKTGFNCDGKLGNESVTFYLQNLYVNQTDIYFCKIEVMAPPPALDNEKSNGTIIHVKGKHLCPSPLFPGPSKPFWVLVVVGGVLACYSLLVTVAFIIFWVRSKRSRGGHSDYMNMTPRRPGPTRKHYQPYAPPRDFAAYRSNCRNTGPWLKKVLKCNTPDPSKFFSQLSSEHGGDVQKWLSSPFPSSSFSPGGLAPEISPLEVLERDKVTQLLPLNTDAYLSLQELQGQDPTHLVRVKFSRSADAPAYQQGQNQLYNELNLGRREEYDVLDKRRGRDPEMGGKPRRKNPQEGLYNELQKDKMAEAYSEIGMKGERRRGKGHDGLYQGLSTATKDTYDAYRHQALPPRGSGSSGEGRGSLLTCGDVEENPGPPVATMVSKGEELFTGVVPILVELDGDVNGHKFSVSGEGEGDATYGKLTLKFICTTGKLPVPWPTLVTTLTYGVQCFSRYPDHMKQHDFFKSAMPEGYVQERTIFFKDDGNYKTRAEVKFEGDTLVNRIELKGIDFKEDGNILGHKLEYNYNSHNVYIMADKQKNGIKVNFKIRHNIEDGSVQLADHYQQNTPIGDGPVLLPDNHYLSTQSALSKDPNEKRDHMVLLEFVTAAGITLGMDELYK

SEQ ID NO: 41 - protein, 1044 aa, synthetic construct
  source 1..1044: note = humanized homo sapiens/mus musculus chimera
MRRMQLLLLIALSLALVTNSEFQVQLVQSGAEVKKPGASVKVSCKASGYTFTHYYIYWVRQAPGQGLEWMGGVNPSNGGTHFNEKFKSRVTMTRDTSISTAYMELSRLRSDDTAVYYCARSEYDYGLGFAYWGQGTLVTVSSGGGGSGGGGSGGGGSDIVMTQSPDSLAVSLGERATINCKSSQSLLNSRTPKNYLAWYQQKPGQPPKLLIYWASTRKSGVPDRFSGSGSGTDFTLTISSLQAEDVAVYYCKQSYNLLTFGGGTKVEIKAAALEKEALKKIIEDQQEALNKWAAAGPGGGGSKILVKQSPMLVAYDNAVNLSCKYSYNLFSREFRASLHKGLDSAVEVCVVYGNYSQQLQVYSKTGFNCDGKLGNESVTFYLQNLYVNQTDIYFCKIEVMAPPPALDNEKSNGTIIHVKGKHLCPSPLFPGPSKPFWVLVVVGGVLACYSLLVTVAFIIFWVRSKRSRGGHSDYMNMTPRRPGPTRKHYQPYAPPRDFAAYRSGGGGSKKRIKPIVWPSLPDHKKTLEHLCKKPRKNLNVSFNPESFLDCQIHRVDDIQARDEVEGFLQDTFPQQLEESEKQRLGGDVQSPNCPSEDVVIGPHVYQDLLLSLGTTNSTLPPPFSLQSGILTLNPVAQGQPILTSLGSNQEEAYVTMSSFYQNQGGGGSFSRSADAPAYQQGQNQLYNELNLGRREEYDVLDKRRGRDPEMGGKPRRKNPQEGLYNELQKDKMAEAYSEIGMKGERRRGKGHDGLYQGLSTATKDTYDALHMQALPPRGSGSSGEGRGSLLTCGDVEENPGPPVATMVSKGEELFTGVVPILVELDGDVNGHKFSVSGEGEGDATYGKLTLKFICTTGKLPVPWPTLVTTLTYGVQCFSRYPDHMKQHDFFKSAMPEGYVQERTIFFKDDGNYKTRAEVKFEGDTLVNRIELKGIDFKEDGNILGHKLEYNYNSHNVYIMADKQKNGIKVNFKIRHNIEDGSVQLADHYQQNTPIGDGPVLLPDNHYLSTQSALSKDPNEKRDHMVLLEFVTAAGITLGMDELYK

SEQ ID NO: 42 - protein, 1044 aa, synthetic construct
  source 1..1044: note = humanized homo sapiens/mus musculus chimera
MRRMQLLLLIALSLALVTNSEFQVQLVQSGAEVKKPGASVKVSCKASGYTFTHYYIYWVRQAPGQGLEWMGGVNPSNGGTHFNEKFKSRVTMTRDTSISTAYMELSRLRSDDTAVYYCARSEYDYGLGFAYWGQGTLVTVSSGGGGSGGGGSGGGGSDIVMTQSPDSLAVSLGERATINCKSSQSLLNSRTPKNYLAWYQQKPGQPPKLLIYWASTRKSGVPDRFSGSGSGTDFTLTISSLQAEDVAVYYCKQSYNLLTFGGGTKVEIKAAALEKEALKKIIEDQQEALNKWAAAGPGGGGSKILVKQSPMLVAYDNAVNLSCKYSYNLFSREFRASLHKGLDSAVEVCVVYGNYSQQLQVYSKTGFNCDGKLGNESVTFYLQNLYVNQTDIYFCKIEVMAPPPALDNEKSNGTIIHVKGKHLCPSPLFPGPSKPFWVLVVVGGVLACYSLLVTVAFIIFWVRSKRSRGGHSDYMNMTPRRPGPTRKHYQPYAPPRDFAAYRSGGGGSFSRSADAPAYQQGQNQLYNELNLGRREEYDVLDKRRGRDPEMGGKPRRKNPQEGLYNELQKDKMAEAYSEIGMKGERRRGKGHDGLYQGLSTATKDTYDALHMQALPPRGGGGSKKRIKPIVWPSLPDHKKTLEHLCKKPRKNLNVSFNPESFLDCQIHRVDDIQARDEVEGFLQDTFPQQLEESEKQRLGGDVQSPNCPSEDVVIGPHVYQDLLLSLGTTNSTLPPPFSLQSGILTLNPVAQGQPILTSLGSNQEEAYVTMSSFYQNQGSGSSGEGRGSLLTCGDVEENPGPPVATMVSKGEELFTGVVPILVELDGDVNGHKFSVSGEGEGDATYGKLTLKFICTTGKLPVPWPTLVTTLTYGVQCFSRYPDHMKQHDFFKSAMPEGYVQERTIFFKDDGNYKTRAEVKFEGDTLVNRIELKGIDFKEDGNILGHKLEYNYNSHNVYIMADKQKNGIKVNFKIRHNIEDGSVQLADHYQQNTPIGDGPVLLPDNHYLSTQSALSKDPNEKRDHMVLLEFVTAAGITLGMDELYK

SEQ ID NO: 43 - protein, 884 aa, synthetic construct
  source 1..884: note = humanized homo sapiens/mus musculus chimera
MRRMQLLLLIALSLALVTNSEFQVQLVQSGAEVKKPGASVKVSCKASGYTFTHYYIYWVRQAPGQGLEWMGGVNPSNGGTHFNEKFKSRVTMTRDTSISTAYMELSRLRSDDTAVYYCARSEYDYGLGFAYWGQGTLVTVSSGGGGSGGGGSGGGGSDIVMTQSPDSLAVSLGERATINCKSSQSLLNSRTPKNYLAWYQQKPGQPPKLLIYWASTRKSGVPDRFSGSGSGTDFTLTISSLQAEDVAVYYCKQSYNLLTFGGGTKVEIKAAALEKEALKKIIEDQQEALNKWAAAGPGGGGSKILVKQSPMLVAYDNAVNLSCKYSYNLFSREFRASLHKGLDSAVEVCVVYGNYSQQLQVYSKTGFNCDGKLGNESVTFYLQNLYVNQTDIYFCKIEVMAPPPALDNEKSNGTIIHVKGKHLCPSPLFPGPSKPFWVLVVVGGVLACYSLLVTVAFIIFWVRSKRSRGGHSDYMFMTPRRPGPTRKHYQPYAPPRDFAAYRSGGGGSFSRSADAPAYQQGQNQLYNELNLGRREEYDVLDKRRGRDPEMGGKPRRKNPQEGLYNELQKDKMAEAYSEIGMKGERRRGKGHDGLYQGLSTATKDTYDALHMQALPPRGSGSSGEGRGSLLTCGDVEENPGPPVATMVSKGEELFTGVVPILVELDGDVNGHKFSVSGEGEGDATYGKLTLKFICTTGKLPVPWPTLVTTLTYGVQCFSRYPDHMKQHDFFKSAMPEGYVQERTIFFKDDGNYKTRAEVKFEGDTLVNRIELKGIDFKEDGNILGHKLEYNYNSHNVYIMADKQKNGIKVNFKIRHNIEDGSVQLADHYQQNTPIGDGPVLLPDNHYLSTQSALSKDPNEKRDHMVLLEFVTAAGITLGMDELYK

SEQ ID NO: 44 - protein, 922 aa, synthetic construct
  source 1..922: note = humanized homo sapiens/mus musculus chimera
MRRMQLLLLIALSLALVTNSEFQVQLVQSGAEVKKPGASVKVSCKASGYTFTHYYIYWVRQAPGQGLEWMGGVNPSNGGTHFNEKFKSRVTMTRDTSISTAYMELSRLRSDDTAVYYCARSEYDYGLGFAYWGQGTLVTVSSGGGGSGGGGSGGGGSDIVMTQSPDSLAVSLGERATINCKSSQSLLNSRTPKNYLAWYQQKPGQPPKLLIYWASTRKSGVPDRFSGSGSGTDFTLTISSLQAEDVAVYYCKQSYNLLTFGGGTKVEIKAAALEKEALKKIIEDQQEALNKWAAAGPGGGGSKILVKQSPMLVAYDNAVNLSCKYSYNLFSREFRASLHKGLDSAVEVCVVYGNYSQQLQVYSKTGFNCDGKLGNESVTFYLQNLYVNQTDIYFCKIEVMAPPPALDNEKSNGTIIHVKGKHLCPSPLFPGPSKPFWLPIGCAAFVVVCILGCILICWLTKKKYSSSVHDPNGEYMFMRAVNTAKKSRLTDVTLGGGGSKRGRKKLLYIFKQPFMRPVQTTQEEDGCSCRFPEEEEGGCELGGGGSFSRSADAPAYQQGQNQLYNELNLGRREEYDVLDKRRGRDPEMGGKPRRKNPQEGLYNELQKDKMAEAYSEIGMKGERRRGKGHDGLYQGLSTATKDTYDALHMQALPPRGSGSSGEGRGSLLTCGDVEENPGPPVATMVSKGEELFTGVVPILVELDGDVNGHKFSVSGEGEGDATYGKLTLKFICTTGKLPVPWPTLVTTLTYGVQCFSRYPDHMKQHDFFKSAMPEGYVQERTIFFKDDGNYKTRAEVKFEGDTLVNRIELKGIDFKEDGNILGHKLEYNYNSHNVYIMADKQKNGIKVNFKIRHNIEDGSVQLADHYQQNTPIGDGPVLLPDNHYLSTQSALSKDPNEKRDHMVLLEFVTAAGITLGMDELYK

SEQ ID NO: 45 - protein, 875 aa, synthetic construct
  source 1..875: note = humanized homo sapiens/mus musculus chimera
MRRMQLLLLIALSLALVTNSEFQVQLVQSGAEVKKPGASVKVSCKASGYTFTHYYIYWVRQAPGQGLEWMGGVNPSNGGTHFNEKFKSRVTMTRDTSISTAYMELSRLRSDDTAVYYCARSEYDYGLGFAYWGQGTLVTVSSGGGGSGGGGSGGGGSDIVMTQSPDSLAVSLGERATINCKSSQSLLNSRTPKNYLAWYQQKPGQPPKLLIYWASTRKSGVPDRFSGSGSGTDFTLTISSLQAEDVAVYYCKQSYNLLTFGGGTKVEIKAAALEKEALKKIIEDQQEALNKWAAAGPGGGGSKILVKQSPMLVAYDNAVNLSCKYSYNLFSREFRASLHKGLDSAVEVCVVYGNYSQQLQVYSKTGFNCDGKLGNESVTFYLQNLYVNQTDIYFCKIEVMAPPPALDNEKSNGTIIHVKGKHLCPSPLFPGPSKPFWLPIGCAAFVVVCILGCILICWLTKKKYSSSVHDPNGEYMFMRAVNTAKKSRLTDVTLGGGGSFSRSADAPAYQQGQNQLYNELNLGRREEYDVLDKRRGRDPEMGGKPRRKNPQEGLYNELQKDKMAEAYSEIGMKGERRRGKGHDGLYQGLSTATKDTYDALHMQALPPRGSGSSGEGRGSLLTCGDVEENPGPPVATMVSKGEELFTGVVPILVELDGDVNGHKFSVSGEGEGDATYGKLTLKFICTTGKLPVPWPTLVTTLTYGVQCFSRYPDHMKQHDFFKSAMPEGYVQERTIFFKDDGNYKTRAEVKFEGDTLVNRIELKGIDFKEDGNILGHKLEYNYNSHNVYIMADKQKNGIKVNFKIRHNIEDGSVQLADHYQQNTPIGDGPVLLPDNHYLSTQSALSKDPNEKRDHMVLLEFVTAAGITLGMDELYK

SEQ ID NO: 46 - protein, 525 aa, synthetic construct
  source 1..525: note = targeting module
EVQLQQSGPELVKPGASVKMSCKASGYTFTDYYMKWVKQSHGKSLEWIGDIIPSNGATFYNQKFKGKATLTVDRSSSTAYMHLNSLTSEDSAVYYCTRSHLLRASWFAYWGQGTLVTVSAASGGGGSGGGGSGGGGSDFVMTQSPSSLTVTAGEKVTMSCKSSQSLLNSGNQKNYLTWYLQKPGQPPKLLIYWASTRESGVPDRFTGSGSGTDFTLTISSVQAEDLAVYYCQNDYSYPYTFGGGTKLEIKAAARGQVQLVQSGAEVKKPGASVKVSCKASGYTFTHYYIYWVRQAPGQGLEWMGGVNPSNGGTHFNEKFKSRVTMTRDTSISTAYMELSRLRSDDTAVYYCARSEYDYGLGFAYWGQGTLVTVSSGGGGSGGGGSGGGGSDIVMTQSPDSLAVSLGERATINCKSSQSLLNSRTPKNYLAWYQQKPGQPPKLLIYWASTRKSGVPDRFSGSGSGTDFTLTISSLQAEDVAVYYCKQSYNLLTFGGGTKVEIKGPEQKLISEEDLNSAVDHHHHHH

SEQ ID NO: 47 - protein, 516 aa, synthetic construct
  source 1..516: note = targeting module
GQVQLVQSGAEVKKPGASVKVSCKASGYTFTDYYMHWVRQAPGQGLEWMGDIIPSNGATFYAQKFQGRVTMTRDTSTSTVYMELSSLRSEDTAVYYCTRSHLLRASWFAYWGQGTLVTVSSASGGGGSGGGGSGGGGSDIVMTQSPDSLAVSLGERATINCKSSQSLLNSGNQKNYLAWYQQKPGQPPKLLIYWASTRESGVPDRFSGSGSGTDFTLTISSLQAEDVAVYYCQNDYSYPYTFGGGTKLEIKAAARGQVQLVQSGAEVKKPGASVKVSCKASGYTFTHYYIYWVRQAPGQGLEWMGGVNPSNGGTHFNEKFKSRVTMTRDTSISTAYMELSRLRSDDTAVYYCARSEYDYGLGFAYWGQGTLVTVSSGGGGSGGGGSGGGGSDIVMTQSPDSLAVSLGERATINCKSSQSLLNSRTPKNYLAWYQQKPGQPPKLLIYWASTRKSGVPDRFSGSGSGTDFTLTISSLQAEDVAVYYCKQSYNLLTFGGGTKVEIKGGGGSHHHHHHHH

SEQ ID NO: 48 - protein, 526 aa, synthetic construct
  source 1..526: note = targeting module
GQVQLVQSGAEVKKPGSSVKVSCKASGYTFTDYYIHWVRQAPGQGLEWMGDIIPSNGATFYNQRFKGRVTITADESTSTAYMELSSLRSEDTAVYYCTRSHLLRASWFAYWGQGTLVTVSSASGGGGSGGGGSGGGGSDIVMTQTPLSLSVTPGQPASISCRSSQSLLNSGNQKNYLTWYLQKPGQSPQLLIYWASTRFIGVPDRFSGSGSGTDFTLKISRVEAEDVGVYYCQNDYSYPYTFGQGTKLEIKAAARGDIVMTQSPDSLAVSLGERATINCKSSQSLLNSRTPKNYLAWYQQKPGQPPKLLIYWASTRKSGVPDRFSGSGSGTDFTLTISSLQAEDVAVYYCKQSYNLLTFGGGTKVEIKGGGGSGGGGSGASAAGGGGSGGGGSQVQLVQSGAEVKKPGASVKVSCKASGYTFTHYYIYWVRQAPGQGLEWMGGVNPSNGGTHFNEKFKSRVTMTRDTSISTAYMELSRLRSDDTAVYYCARSEYDYGLGFAYWGQGTLVTVSSGGGGSHHHHHHHH

SEQ ID NO: 49 - protein, 526 aa, synthetic construct
  source 1..526: note = targeting module
GQVQLVQSGAEVKKPGASVKMSCKASGYTFTDYYMKWVKQAPGQGLEWIGDIIPSNGATFYNQKFQGRATLTVDTSTSTAYMELSSLRSEDTAVYYCTRSHLLRASWFAYWGQGTLVTVSSASGGGGSGGGGSGGGGSDIVMTQSPDSLAVSLGERATINCKSSQSLLNSGNQKNYLTWYLQKPGQPPKLLIYWASTRESGVPDRFSGSGSGTDFTLTISSVQAEDVAVYYCQNDYSYPYTFGGGTKLEIKAAARGDIVMTQSPDSLAVSLGERVTMNCKSSQSLLNSRTPKNYLAWYQQKPGQSPKLLIYWASTRKSGVPDRFSGSGSGTDFTLTISSVQAEDVAVYYCKQSYNLLTFGGGTKLEIKGGGGSGGGGSGASAAGGGGSGGGGSQVQLVESGAEVVKPGASVKLSCKASGYAFTHYYIYWIKQAPGQGLEWIGGVNPSNGGTHFNEKFKSRATLTVDTSISTAYMELSRLRSDDTAVYYCTRSEYDYGLGFAYWGQGTLVTVSSGGGGSHHHHHHHH

SEQ ID NO: 50 - protein, 515 aa, synthetic construct
  source 1..515: note = targeting module
EVQLQQSGPELVKPGASVKMSCKASGYTFTDYYMKWVKQSHGKSLEWIGDIIPSNGATFYNQKFKGKATLTVDRSSSTAYMHLNSLTSEDSAVYYCTRSHLLRASWFAYWGQGTLVTVSAASGGGGSGGGGSGGGGSDFVMTQSPSSLTVTAGEKVTMSCKSSQSLLNSGNQKNYLTWYLQKPGQPPKLLIYWASTRESGVPDRFTGSGSGTDFTLTISSVQAEDLAVYYCQNDYSYPYTFGGGTKLEIKAAARGQVQLVQSGAEVKKPGASVKVSCKASGYTFTHYYIYWVRQAPGQGLEWMGGVNPSNGGTHFNEKFKSRVTMTRDTSISTAYMELSRLRSDDTAVYYCARSEYDYGLGFAYWGQGTLVTVSSGGGGSGGGGSGGGGSDIVMTQSPDSLAVSLGERATINCKSSQSLLNSRTPKNYLAWYQQKPGQPPKLLIYWASTRKSGVPDRFSGSGSGTDFTLTISSLQAEDVAVYYCKQSYNLLTFGGGTKVEIKGGGGSHHHHHHHH

SEQ ID NO: 51 - protein, 525 aa, synthetic construct
  source 1..525: note = targeting module
EVQLQQSGPELVKPGASVKMSCKASGYTFTDYYMKWVKQSHGKSLEWIGDIIPSNGATFYNQKFKGKATLTVDRSSSTAYMHLNSLTSEDSAVYYCTRSHLLRASWFAYWGQGTLVTVSAASGGGGSGGGGSGGGGSDFVMTQSPSSLTVTAGEKVTMSCKSSQSLLNSGNQKNYLTWYLQKPGQPPKLLIYWASTRESGVPDRFTGSGSGTDFTLTISSVQAEDLAVYYCQNDYSYPYTFGGGTKLEIKAAARGDIVMTQSPDSLAVSLGERATINCKSSQSLLNSRTPKNYLAWYQQKPGQPPKLLIYWASTRKSGVPDRFSGSGSGTDFTLTISSLQAEDVAVYYCKQSYNLLTFGGGTKVEIKGGGGSGGGGSGASAAGGGGSGGGGSQVQLVQSGAEVKKPGASVKVSCKASGYTFTHYYIYWVRQAPGQGLEWMGGVNPSNGGTHFNEKFKSRVTMTRDTSISTAYMELSRLRSDDTAVYYCARSEYDYGLGFAYWGQGTLVTVSSGGGGSHHHHHHHH

SEQ ID NO: 52 - protein, 525 aa, synthetic construct
  source 1..525: note = targeting module
EVQLQQSGPELVKPGASVKMSCKASGYTFTDYYMKWVKQSHGKSLEWIGDIIPSNGATFYNQKFKGKATLTVDRSSSTAYMHLNSLTSEDSAVYYCTRSHLLRASWFAYWGQGTLVTVSAASGGGGSGGGGSGGGGSDFVMTQSPSSLTVTAGEKVTMSCKSSQSLLNSGNQKNYLTWYLQKPGQPPKLLIYWASTRESGVPDRFTGSGSGTDFTLTISSVQAEDLAVYYCQNDYSYPYTFGGGTKLEIKAAARGDIVMTQSPDSLAVSLGERVTMNCKSSQSLLNSRTPKNYLAWYQQKPGQSPKLLIYWASTRKSGVPDRFSGSGSGTDFTLTISSVQAEDVAVYYCKQSYNLLTFGGGTKLEIKGGGGSGGGGSGASAAGGGGSGGGGSQVQLVESGAEVVKPGASVKLSCKASGYAFTHYYIYWIKQAPGQGLEWIGGVNPSNGGTHFNEKFKSRATLTVDTSISTAYMELSRLRSDDTAVYYCTRSEYDYGLGFAYWGQGTLVTVSSGGGGSHHHHHHHH

SEQ ID NO: 53 - protein, 516 aa, synthetic construct
  source 1..516: note = targeting module
GQVQLVQSGAEVKKPGSSVKVSCKASGYTFTDYYIHWVRQAPGQGLEWMGDIIPSNGATFYNQRFKGRVTITADESTSTAYMELSSLRSEDTAVYYCTRSHLLRASWFAYWGQGTLVTVSSASGGGGSGGGGSGGGGSDIVMTQTPLSLSVTPGQPASISCRSSQSLLNSGNQKNYLTWYLQKPGQSPQLLIYWASTRFIGVPDRFSGSGSGTDFTLKISRVEAEDVGVYYCQNDYSYPYTFGQGTKLEIKAAARGQVQLVQSGAEVKKPGASVKVSCKASGYTFTHYYIYWVRQAPGQGLEWMGGVNPSNGGTHFNEKFKSRVTMTRDTSISTAYMELSRLRSDDTAVYYCARSEYDYGLGFAYWGQGTLVTVSSGGGGSGGGGSGGGGSDIVMTQSPDSLAVSLGERATINCKSSQSLLNSRTPKNYLAWYQQKPGQPPKLLIYWASTRKSGVPDRFSGSGSGTDFTLTISSLQAEDVAVYYCKQSYNLLTFGGGTKVEIKGGGGSHHHHHHHH

SEQ ID NO: 54 - protein, 516 aa, synthetic construct
  source 1..516: note = targeting module
GQVQLVQSGAEVKKPGASVKMSCKASGYTFTDYYMKWVKQAPGQGLEWIGDIIPSNGATFYNQKFQGRATLTVDTSTSTAYMELSSLRSEDTAVYYCTRSHLLRASWFAYWGQGTLVTVSSASGGGGSGGGGSGGGGSDIVMTQSPDSLAVSLGERATINCKSSQSLLNSGNQKNYLTWYLQKPGQPPKLLIYWASTRESGVPDRFSGSGSGTDFTLTISSVQAEDVAVYYCQNDYSYPYTFGGGTKLEIKAAARGQVQLVQSGAEVKKPGASVKVSCKASGYTFTHYYIYWVRQAPGQGLEWMGGVNPSNGGTHFNEKFKSRVTMTRDTSISTAYMELSRLRSDDTAVYYCARSEYDYGLGFAYWGQGTLVTVSSGGGGSGGGGSGGGGSDIVMTQSPDSLAVSLGERATINCKSSQSLLNSRTPKNYLAWYQQKPGQPPKLLIYWASTRKSGVPDRFSGSGSGTDFTLTISSLQAEDVAVYYCKQSYNLLTFGGGTKVEIKGGGGSHHHHHHHH

SEQ ID NO: 55 - protein, 526 aa, synthetic construct
  source 1..526: note = targeting module
GQVQLVQSGAEVKKPGASVKMSCKASGYTFTDYYMKWVKQAPGQGLEWIGDIIPSNGATFYNQKFQGRATLTVDTSTSTAYMELSSLRSEDTAVYYCTRSHLLRASWFAYWGQGTLVTVSSASGGGGSGGGGSGGGGSDIVMTQSPDSLAVSLGERATINCKSSQSLLNSGNQKNYLTWYLQKPGQPPKLLIYWASTRESGVPDRFSGSGSGTDFTLTISSVQAEDVAVYYCQNDYSYPYTFGGGTKLEIKAAARGDIVMTQSPDSLAVSLGERATINCKSSQSLLNSRTPKNYLAWYQQKPGQPPKLLIYWASTRKSGVPDRFSGSGSGTDFTLTISSLQAEDVAVYYCKQSYNLLTFGGGTKVEIKGGGGSGGGGSGASAAGGGGSGGGGSQVQLVQSGAEVKKPGASVKVSCKASGYTFTHYYIYWVRQAPGQGLEWMGGVNPSNGGTHFNEKFKSRVTMTRDTSISTAYMELSRLRSDDTAVYYCARSEYDYGLGFAYWGQGTLVTVSSGGGGSHHHHHHHH

SEQ ID NO: 56 - protein, 526 aa, synthetic construct
  source 1..526: note = targeting module
GQVQLVQSGAEVKKPGASVKMSCKASGYTFTDYYMKWVKQAPGQGLEWIGDIIPSNGATFYNQKFKGRATLTVDKSTSTAYMELSSLRSEDTAVYYCTRSHLLRASWFAYWGQGTLVTVSSASGGGGSGGGGSGGGGSDFVMTQSPDSLAVSLGERATMNCKSSQSLLNSGNQKNYLTWYLQKPGQPPKLLIYWASTRESGVPDRFSGSGSGTDFTLTISSVQAEDVAVYYCQNDYSYPYTFGGGTKLEIKAAARGQVQLVQSGAEVKKPGASVKVSCKASGYTFTHYYIYWVRQAPGQGLEWMGGVNPSNGGTHFNEKFKSRVTMTRDTSISTAYMELSRLRSDDTAVYYCARSEYDYGLGFAYWGQGTLVTVSSGGGGSGGGGSGASAAGGGGSGGGGSDIVMTQSPDSLAVSLGERATINCKSSQSLLNSRTPKNYLAWYQQKPGQPPKLLIYWASTRKSGVPDRFSGSGSGTDFTLTISSLQAEDVAVYYCKQSYNLLTFGGGTKVEIKGGGGSHHHHHHHH

SEQ ID NO: 57 - protein, 526 aa, synthetic construct
  source 1..526: note = targeting module
GQVQLVQSGAEVKKPGASVKMSCKASGYTFTDYYMKWVKQAPGQGLEWIGDIIPSNGATFYNQKFKGRATLTVDKSTSTAYMELSSLRSEDTAVYYCTRSHLLRASWFAYWGQGTLVTVSSASGGGGSGGGGSGGGGSDFVMTQSPDSLAVSLGERATMNCKSSQSLLNSGNQKNYLTWYLQKPGQPPKLLIYWASTRESGVPDRFSGSGSGTDFTLTISSVQAEDVAVYYCQNDYSYPYTFGGGTKLEIKAAARGDIVMTQSPDSLAVSLGERATINCKSSQSLLNSRTPKNYLAWYQQKPGQPPKLLIYWASTRKSGVPDRFSGSGSGTDFTLTISSLQAEDVAVYYCKQSYNLLTFGGGTKVEIKGGGGSGGGGSGASAAGGGGSGGGGSQVQLVQSGAEVKKPGASVKVSCKASGYTFTHYYIYWVRQAPGQGLEWMGGVNPSNGGTHFNEKFKSRVTMTRDTSISTAYMELSRLRSDDTAVYYCARSEYDYGLGFAYWGQGTLVTVSSGGGGSHHHHHHHH

SEQ ID NO: 58 - protein, 525 aa, synthetic construct
  source 1..525: note = targeting module
EVQLVQSGAEVKKPGASVKMSCKASGYTFTDYYMKWVKQAPGQGLEWIGDIIPSNGATFYNQKFKGRATLTVDRSTSTAYMELSSLRSEDTAVYYCTRSHLLRASWFAYWGQGTLVTVSSASGGGGSGGGGSGGGGSDFVMTQSPDSLAVSLGERATINCESSQSLLNTGNQKNYLTWYLQKPGQPPKLLIYWASTRESGVPDRFSGSGSGTDFTLTISSVQAEDVAVYYCQNDYSYPYTFGGGTKLEIKAAARGDIVMTQSPDSLAVSLGERATINCKSSQSLLNSRTPKNYLAWYQQKPGQPPKLLIYWASTRKSGVPDRFSGSGSGTDFTLTISSLQAEDVAVYYCKQSYNLLTFGGGTKVEIKGGGGSGGGGSGASAAGGGGSGGGGSQVQLVQSGAEVKKPGASVKVSCKASGYTFTHYYIYWVRQAPGQGLEWMGGVNPSNGGTHFNEKFKSRVTMTRDTSISTAYMELSRLRSDDTAVYYCARSEYDYGLGFAYWGQGTLVTVSSGGGGSHHHHHHHH

SEQ ID NO: 59 - protein, 525 aa, synthetic construct
  source 1..525: note = targeting module
EVQLVQSGAEVKKPGASVKMSCKASGYTFTDYYMKWVKQAPGQGLEWIGDIIPSNGATFYNQKFKGRATLTVDRSTSTAYMELSSLRSEDTAVYYCTRSHLLRASWFAYWGQGTLVTVSSASGGGGSGGGGSGGGGSDFVMTQSPDSLAVSLGERATINCESSQSLLNTGNQKNYLTWYLQKPGQPPKLLIYWASTRESGVPDRFSGSGSGTDFTLTISSVQAEDVAVYYCQNDYSYPYTFGGGTKLEIKAAARGDIVMTQSPDSLAVSLGERVTMNCKSSQSLLNSRTPKNYLAWYQQKPGQSPKLLIYWASTRKSGVPDRFSGSGSGTDFTLTISSVQAEDVAVYYCKQSYNLLTFGGGTKLEIKGGGGSGGGGSGASAAGGGGSGGGGSQVQLVESGAEVVKPGASVKLSCKASGYAFTHYYIYWIKQAPGQGLEWIGGVNPSNGGTHFNEKFKSRATLTVDTSISTAYMELSRLRSDDTAVYYCTRSEYDYGLGFAYWGQGTLVTVSSGGGGSHHHHHHHH

SEQ ID NO: 60 - protein, 468 aa, synthetic construct
  source 1..468: note = humanized homo sapiens/mus musculus chimera
MRRMQLLLLIALSLALVTNSEFKPLPEVTDEYAAAGPGGGGSKILVKQSPMLVAYDNAVNLSCKYSYNLFSREFRASLHKGLDSAVEVCVVYGNYSQQLQVYSKTGFNCDGKLGNESVTFYLQNLYVNQTDIYFCKIEVMAPPPALDNEKSNGTIIHVKGKHLCPSPLFPGPSKPFWVLVVVGGVLACYSLLVTVAFIIFWVGGSSGEGRGSLLTCGDVEENPGPPVATMVSKGEELFTGVVPILVELDGDVNGHKFSVSGEGEGDATYGKLTLKFICTTGKLPVPWPTLVTTLTYGVQCFSRYPDHMKQHDFFKSAMPEGYVQERTIFFKDDGNYKTRAEVKFEGDTLVNRIELKGIDFKEDGNILGHKLEYNYNSHNVYIMADKQKNGIKVNFKIRHNIEDGSVQLADHYQQNTPIGDGPVLLPDNHYLSTQSALSKDPNEKRDHMVLLEFVTAAGITLGMDELYK

SEQ ID NO: 61 - protein, 728 aa, synthetic construct
  source 1..728: note = humanized homo sapiens/mus musculus chimera
MRRMQLLLLIALSLALVTNSEFQVQLVQSGAEVKKPGASVKVSCKASGYTFTHYYIYWVRQAPGQGLEWMGGVNPSNGGTHFNEKFKSRVTMTRDTSISTAYMELSRLRSDDTAVYYCARSEYDYGLGFAYWGQGTLVTVSSGGGGSGGGGSGGGGSDIVMTQSPDSLAVSLGERATINCKSSQSLLNSRTPKNYLAWYQQKPGQPPKLLIYWASTRKSGVPDRFSGSGSGTDFTLTISSLQAEDVAVYYCKQSYNLLTFGGGTKVEIKAAALEKEALKKIIEDQQEALNKWAAAGPGGGGSKILVKQSPMLVAYDNAVNLSCKYSYNLFSREFRASLHKGLDSAVEVCVVYGNYSQQLQVYSKTGFNCDGKLGNESVTFYLQNLYVNQTDIYFCKIEVMAPPPALDNEKSNGTIIHVKGKHLCPSPLFPGPSKPFWVLVVVGGVLACYSLLVTVAFIIFWVGGSSGEGRGSLLTCGDVEENPGPPVATMVSKGEELFTGVVPILVELDGDVNGHKFSVSGEGEGDATYGKLTLKFICTTGKLPVPWPTLVTTLTYGVQCFSRYPDHMKQHDFFKSAMPEGYVQERTIFFKDDGNYKTRAEVKFEGDTLVNRIELKGIDFKEDGNILGHKLEYNYNSHNVYIMADKQKNGIKVNFKIRHNIEDGSVQLADHYQQNTPIGDGPVLLPDNHYLSTQSALSKDPNEKRDHMVLLEFVTAAGITLGMDELYK